European Patent Application EP 4 570 918 A1, published June 18, 2025. Title: 一种双荧光素酶报告基因检测系统及其应用. Applicant: 深圳华大生命科学研究院. The sequence listing filed with the application follows.

SEQUENCE LISTING (9 sequences)

SEQ ID NO: 1 - protein, 168 aa, synthetic construct
KPTENNEDFNIVAVASNFATTDLDADRGKLPGKKLPLEVLKEMEANARKAGCTRGCLICLSHIKCTPKMKKFIPGRCHTYEGDKESAQGGIGEAIVDIPEIPGFKDLEPMEQFIAQVDLCVDCTTGCLKGLANVQCSDLLKKWLPQRCATFASKIQGQVDKIKGAGGD

SEQ ID NO: 2 - DNA, 504 bp, synthetic construct
  source 1..504: mol_type = other DNA
aaaccaactgaaaacaatgaagatttcaacattgtagctgtagctagcaactttgctacaacggatctcgatgctgaccgtggtaaattgcccggaaaaaaattaccacttgaggtactcaaagaaatggaagccaatgctaggaaagctggctgcactaggggatgtctgatatgcctgtcacacatcaagtgtacacccaaaatgaagaagtttatcccaggaagatgccacacctatgaaggagacaaagaaagtgcacagggaggaataggagaggctattgttgacattcctgaaattcctgggtttaaggatttggaacccatggaacaattcattgcacaagttgacctatgtgtagactgcacaactggatgcctcaaaggtcttgccaatgtgcaatgttctgatttactcaagaaatggctgccacaaagatgtgcaacttttgctagcaaaattcaaggccaagtggacaaaataaagggtgccggtggtgat

SEQ ID NO: 3 - protein, 163 aa, Pleuromamma xiphias
QPTENKQESHIVDSDLDGDRGRKLPGKKLPIEVLKIMEANARRAGCTRGCLICLSKIKCTAKMKRYIPGRCHTYEGDKSIGQGGIGGPIVDIPEIIGFKNMEPMDQFIAQVDLCADCTTGCLKGLANVRCNDLLKKWLPDRCAGFADKIQNEVDSIKGMAGDR

SEQ ID NO: 4 - protein, 180 aa, synthetic construct
MYIKVWFGLACLSLVLAOPTENKOESHIVDSDLDGDRGRKLPGKKLPIEVLKIMEANARRAGCTRGCLICLSKIKCTAKMKRYIPGRCHTYEGDKSIGOGGIGGPIVDIPEIIGFKNMEPMDOFIAOVDLCADCTTGCLKGLANVRCNDLLKKWLPDRCAGFADKIQNEVDSIKGMAGDR

SEQ ID NO: 5 - DNA, 489 bp, Pleuromamma xiphias
  source 1..489: mol_type = other DNA
caaccaactgaaaacaagcaggagtctcatattgtagattcagatcttgatggcgaccgtggtaggaagttgcccggaaaaaagcttcctatagaagtactcaaaatcatggaagccaatgccaggagagctggttgcactagaggatgtctcatatgtctttcaaaaatcaagtgtacagccaaaatgaagcgatacattccagggagatgtcatacttatgaaggagataaatctattggacagggaggcataggtggccctattgttgatattcctgaaattattggattcaagaacatggaacccatggatcagttcatcgcacaagttgatctgtgcgccgactgtacaactgggtgcctgaaaggccttgctaatgttaggtgcaatgacttgctgaagaaatggctgcctgacagatgtgctggttttgccgacaaaattcaaaatgaagtggatagtatcaagggcatggctggggatcgc

SEQ ID NO: 6 - DNA, 507 bp, synthetic construct
  source 1..507: mol_type = other DNA
atgaaaccaactgaaaacaatgaagatcgcaacattttcgctgtagttgagaactttgttacgacggatattgatgctgaccgtggtaaattgcccggaaaaaaattaccacttgaggtactcaaagaaatggaagccaatgctaggcctgctggctgcactaggggatgtctgatatgcctgtcaaaaatcaagtgtacactcaaaatgaagaagtttatcccaggaagatgccacacctatgaaggagacaaatcaactggacagggaggaataggaccggctattgttgacattcctgaaattcctgggtttaaggatatggaacccatggaacaattcattgcacaagttgacctatgtgaagactgcacaactggatgcctcaaaggtcttgccaatgtgcaatgttctgatttactcaagaaatggctgccacaaagatgtgcaacttttgctagcaaaattcaaggccaagtggacaaaataaagggtgccggtggtgat

SEQ ID NO: 7 - DNA, 507 bp, synthetic construct
  source 1..507: mol_type = other DNA
atgaaaccaactgaaaacaataaagatttcaacattgtagctgtagctagcaactttgctacaacggatctcgatgctgaccgtggtaaattgcccggaaaaaaattaccacttgaggtactcaaagaaatggaagccaatgctaggaaagctggctgcactaggggatgtctgatatgcctgtcaaaaatcaagtgtacactcaaaatgaagaagtttatcccaggaagatgccacacctatgaaggagacaaatcaactggacagggaggaataggaccggctattgttgacattcctgaaattcctgggtttaaggatggggaacccatggaacaattcattgcacaagttgacctatgtgtagactgcacaactggatgcctcaaaggtcttgccaatgtgcgatgttctgatttactcaagaaatggctgccagacagatgtgcaacttttgctaacaaaattcaaggcgaagtggacacaataaagggtatgaacggtgat

SEQ ID NO: 8 - DNA, 507 bp, synthetic construct
  source 1..507: mol_type = other DNA
atgaaaccaactgaaaacaatgaagatttcaacattgtagctgtagctagcaactttgctacaacggatctcgatgctgaccgtggtaaattgcccggaaaaaaattaccacttgaggtactcaaagaaatggaagccaatgctaggaaagctggctgcactaggggatgtctgatatgcctgtcaaaaatcaagtgtacactcaaaatgaagaagtttatcccaggaagatgccacacctatgaaggagacaaatcaactggacagggaggaataggaccggctattgttgacattcctgaaattcctgggtttaaggatatggaacccatggaacaattcattgcacaagttgacctatgtgtagactgcacaactggatgcctcaaaggtcttgccaatgtgcattgttctgatttactcaagaaatggctgccagacagatgtgcaagttttgctaccaaaattcaaaagcaagtggacaaaataaagggtatggctggtgat

SEQ ID NO: 9 - DNA, 489 bp, synthetic construct
  source 1..489: mol_type = other DNA
caaccaactgaaaacaagcaggagtctcatattgtagattcagatcttgatggcgaccgtggtaggaagttgcccggaaaaaagcttcctatagaagtactcaaaatcatggaagccaatgccaggagagctggttgcactagaggatgtctcatatgtctttcaaaaatcaagtgtacagccaaaatgaagcgatacattccagggagatgtcatacttatgaaggagataaatctattggacaggcaccgataggtggccctattgttgatattcctgaaattattggattcaagaacatggaacccatggatcagttcatcgcacaagttgatctgtgcgccgactgtacaactgggtgcctgaaaggccttgctaatgttaggtgcaatgacttgctgaagaaatggctgcctgacagatgtgctggttttgccgacaaaattcaaaatgaagtggatagtatcaagggcatggctggggatcgc